European Patent Application EP 4 446 415 A1, published October 16, 2024. Title: NUCLEIC ACID MOLECULE AND USE OF THE NUCLEIC ACID MOLECULE IN THERAPY OF DISEASES INDUCED BY EXPANSION OF TRINUCLEOTIDE CAG REPEATS. Applicant: Dystrogen Gene Therapies Inc. The sequence listing filed with the application follows.

SEQUENCE LISTING (8 sequences)

SEQ ID NO: 1 - RNA, 21 nt, synthetic construct
  source 1..21: mol_type = other RNA
gctgctgcagcagctgctgct

SEQ ID NO: 2 - RNA, 21 nt, synthetic construct
  source 1..21: mol_type = other RNA
gctgctgcagctggtgctgct

SEQ ID NO: 3 - RNA, 21 nt, synthetic construct
  source 1..21: mol_type = other RNA
gctgctgcagctgatgctgct

SEQ ID NO: 4 - RNA, 21 nt, synthetic construct
  source 1..21: mol_type = other RNA
gctgctgcagctggtgttgct

SEQ ID NO: 5 - RNA, 155 nt, synthetic construct
  source 1..155: mol_type = other RNA
cactccactgcccgacgtcgcctcggtggtgttggatgagccctcggagctgctgcagctgatgctgctggattcttatgctccagcagcatcagctgcagcagttcagagggttctatcatttcgtcggatggaaaggagtgtattctgaagat

SEQ ID NO: 6 - RNA, 155 nt, synthetic construct
  source 1..155: mol_type = other RNA
cactccactgcccgacgtcgcctcggtggtgttggatgagccctcggagctgctgcagcagctgctgctggattcttatgctccagcagcatctgctgcagcagttcagagggttctatcatttcctcggatggaaaggagtgtattctgaagat

SEQ ID NO: 7 - RNA, 155 nt, synthetic construct
  source 1..155: mol_type = other RNA
cactccactgcccgacgtcgcctcggtggtgttggatgagccctcggagctgctgcagctggtgctgctggattcttatgctccagcagcaccagctgcagcagttcagagggttctatcatttcgtcggatggaaaggagtgtattctgaagat

SEQ ID NO: 8 - RNA, 155 nt, synthetic construct
  source 1..155: mol_type = other RNA
cactccactgcccgacgtcgcctcggtggtgttggatgagccctcggagctgctgcagctggtgttgctggattcttatgctccagcaacaccagctgcagcagttcagagggttctatcatttcgtcggatggaaaggagtgtattctgaagat